European Patent Application EP 4 293 117 A1, published December 20, 2023. Title: Uricase activator and uric acid measuring agent. Applicant: Oriental Yeast Co., Ltd. The sequence listing filed with the application follows.

SEQUENCE LISTING (14 sequences)

SEQ ID NO: 1 - protein, 118 aa, Mus musculus
MATESSPLTTHVLDTASGLPAQGLCLRLSRLEAPCQQWMELRTSYTNLDGRCPGLLTPSQIKPGTYKLFFDTERYWKERGQESFYPYVEVVFTITKETQKFHVPLLLSPWSYTTYRGS

SEQ ID NO: 2 - protein, 119 aa, Branchiostoma japonicum
MSANRTSPITTHILDTSLGRPAADVPIKLYRRAERIGQEWSQVSSGQTNSDGRCNGLLNSLEAGVYKITFETATYFNKNGIRQYFYPYVDIVFEIQDPIQHYHVPLLLNPFGYSTYRGS

SEQ ID NO: 3 - protein, 119 aa, Danio renio
MAATLLSPLSTHVLNIAQGVPGANMTIVLHRLDPVSSAWNILTTGITNDDGRCPGLITKENFIAGVYKMRFETGKYWDALGETCFYPYVEIVFTITNTSQHYHVPLLLSRFSYSTYRGS

SEQ ID NO: 4 - protein, 118 aa, Oncorhynchus kisutch
MAAPYSPLTTHVLNTGMGVPGAHMALSLHRMDPSTSLWNLLTTGTTNDDGRCPGLITRETFTPAVYKIRFETGQYWGSLGETSFYPYVEIVFTITDHSQKFHVPLLCSRFSYTTYRGS

SEQ ID NO: 5 - protein, 528 aa, Glycine max
DNYSRDDFPLDFVFGSGTSAYQVEGAANKDGRTPSIWDTFAYAGYAHGENGDVACDGYHKYKEDVQLMLETGLDAYRFSISWSRLLPNGRGPVNPKGLQYSNNLINELISNGIQPHATLYNFDLPQVLEDEYGGWISRDIIRDFTYYAEVEFREFGDRVLYWTTVNEPNVFALGGYDQGNSPPRRCSPPFCATNDTMGNSTYEPYLAVHHILLSHSSAARLYWRKYRDKQHGFVGISIYTFGIFPQTNTEKDRVASQRARDFFVGWIMEPLQYGDYPISMKTNAGERIPAFTNHESKQVKGSFDFIGVIHYTNLNVSDNSDALKNQLRDFTADMAANIFGEDLFSNEEYLITPWGLRQELNKFKLLYGNPPIFIHENGQRTASNSSLQDVDKGEILHGYIGSVLDALRDASNIKGYFRMAFPGFVRVARWIQVSFGLYYVDRDDPQLKKIPKLFCKNGTTGFLKGRRTSILDLFELEQDPITCSKSPIIFSKISKWVLASLLFLIQHKIKFMWREPLPGQIPLKLVMF

SEQ ID NO: 6 - protein, 324 aa, Arabidopsis thaliana
MAMEIGEDEWKVCCGSSEFAKQMSTSGPLTSQEAIYTARDIWFNQVNVTDWLEAFSAHPQIGNTPSPSINSDFARRSVSEQSTAFATTSASALQELAEWNVLYKKKFGFIFIICASGRTHAEMLHALKERYENRPIVELEIAAMEQMKITELRMAKLFSDKAKVISETDSSSSPVSTKPQDRLRIIGGHLNVAAEAKAPKRSRPPITTHVLDVSRGAPAAGVEVHLEVWSGTTGPSFVHGGGGVWSSVGTSATDRDGRSGPLMDLVDALNPGTYRISFDTAKYSPGCFFPYVSIVFQVTESQKWEHFHVPLLLAPFSFSTYRGS

SEQ ID NO: 7 - protein, 114 aa, Escherichia coli
AQQNILSVHILNQQTGKPAADVTVTLEKKADNGWLQLNTAKTDKDGRIKALWPEQTATTGDYRVVFKTGDYFKKQNLESFFPEIPVEFHINKVNEHYHVPLLLSQYGYSTYRGS

SEQ ID NO: 8 - protein, 114 aa, Bacillus subtilis
MGKLTTHILDLTCGKPAANVKIGLKRLGESIMKEVYTNNDGRVDVPLLAGEELMSGEYVMEFHAGDYFASKNMNAADQPFLTIVTVRFQLADPDAHYHIPLLLSPFGYQVYRGS

SEQ ID NO: 9 - protein, 117 aa, Herbaspirillum sp.
MGKLSTHVLDITKGKPGVGVKLALYAVGPVGKTLLKQAVTNSDGRCDEPLLAGEALQVGKYELVFAAGDYFAAQGEQLPEPRFVDEVVIAFGIADASQNYHVPLVVSPWAYSTYRGS

SEQ ID NO: 10 - protein, 119 aa, Deinococcus radiodurans
MSGHPGLTTHVLDTARGKPAAGVRVQLCRVTGDTRTPVTEAVTNSDGRTDAPLIERGSLKQGTYELTFHVADYFKGFVAAADPPFLDVVTLRFTVGDTSGHYHVPLVMTPWSYSTYRGS

SEQ ID NO: 11 - protein, 108 aa, Klebsiella pneumoniae
MSTLSTHILDISTGTPAEGVTVSLSREGETLANLVTNAQGRIATFSAAPLPAGRYCLTAETGAWFARAGRESVFTRAQIDFVIGEAAEDHFHLPFLIAPGGWSTYRGS

SEQ ID NO: 12 - protein, 114 aa, Salmonella enterica
AGNNILSVHILDQQTGKPAPGVEVVLEQKKDNGWTQLNTGHTDQDGRIKALWPEKAAAPGDYRVIFKTGQYFESKKLDTFFPEIPVEFHISKTNEHYHVPLLLSQYGYSTYRGS

SEQ ID NO: 13 - protein, 147 aa, Homo sapiens
MASHRLLLLCLAGLVFVSEAGPTGTGESKCPLMVKVLDAVRGSPAINVAVHVFRKAADDTWEPFASGKTSESGELHGLTTEEEFVEGIYKVEIDTKSYWKALGISPFHEHAEVVFTANDSGPRRYTIAALLSPYSYSTTAVVTNPKE

SEQ ID NO: 14 - protein, 332 aa, Bacillus subtilis
MTKHKERVMYYGKGDVFAYRTYLKPLTGVRTIPESPFSGRDHILFGVNVKISVGGTKLLTSFTKGDNSLVVATDSMKNFIQKHLASYTGTTIEGFLEYVATSFLKKYSHIEKISLIGEEIPFETTFAVKNGNRAASELVFKKSRNEYATAYLNMVRNEDNTLNITEQQSGLAGLQLIKVSGNSFVGFIRDEYTTLPEDSNRPLFVYLNIKWKYKNTEDSFGTNPENYVAAEQIRDIATSVFHETETLSIQHLIYLIGRRILERFPQLQEVYFESQNHTWDKIVEEIPESEGKVYTEPRPPYGFQCFTVTQEDLPHENILMFSDEPDHKGALK